European Patent Application EP 4 119 193 A1, published January 18, 2023. Title: A method for culturing cells derived from epithelial tissue and a composition comprising cells cultured by the method. Applicant: JBM Incorporation GN Corporation Ltd. The sequence listing filed with the application follows.

SEQUENCE LISTING (4 sequences)

SEQ ID NO: 1 - DNA, 20 bp, Artificial Sequence
  Forward primer for GAPDH
gcaccgtcaaggctgagaac

SEQ ID NO: 2 - DNA, 19 bp, Artificial Sequence
  Reverse primer for GAPDH
tggtgaagacgccagtgga

SEQ ID NO: 3 - DNA, 23 bp, Artificial Sequence
  Forward primer for CK3
gggaacagatcaagaccctcaac

SEQ ID NO: 4 - DNA, 22 bp, Artificial Sequence
  Reverse primer for CK3
tgtgcctgagatggaacttgtg